European Patent Specification EP 3 787 664 B1, published February 28, 2024. Title: PEPTIDE HYDROGELS FOR DELIVERY OF IMMUNOSUPPRESSIVE DRUGS AND USES THEREOF. Applicant: THE UNITED STATES OF AMERICA, AS REPRESENTED BY THE SECRETARY, DEPARTMENT OF HEALTH AND HUMAN SERVICES THE JOHNS HOPKINS UNIVERSITY. The sequence listing filed with the application follows.

SEQUENCE LISTING (2 sequences)

SEQ ID NO: 1 - protein, 24 aa, Artificial Sequence
  Synthetic peptide
  misc_feature (1)..(1): Xaa can be any one of F, I, L, M, T, V, W, and Y, or is not present
  misc_feature (2)..(2): Xaa can be any amino acid, or is not present if X1 is not present
  misc_feature (3)..(3): Xaa can be any one of F, I, L, M, T, V, W, and Y, or is not present
  misc_feature (4)..(4): Xaa can be any amino acid, or is not present if X3 is not present
  misc_feature (5)..(5): Xaa can be any one of F, I, L, M, T, V, W, and Y
  misc_feature (6)..(6): Xaa can be any amino acid
  misc_feature (7)..(7): Xaa can be any one of F, I, L, M, T, V, W, and Y
  misc_feature (8)..(8): Xaa can be any amino acid
  misc_feature (9)..(9): Xaa can be any one of F, I, L, M, T, V, W, and Y
  misc_feature (10)..(10): Xaa can be any amino acid
  misc_feature (11)..(11): Xaa can be any one of F, I, L, M, T, V, W, and Y
  misc_feature (14)..(14): Xaa can be any one of F, I, L, M, T, V, W, and Y
  misc_feature (15)..(15): Xaa can be any amino acid
  misc_feature (16)..(16): Xaa can be any one of F, I, L, M, T, V, W, and Y
  misc_feature (17)..(17): Xaa can be any amino acid
  misc_feature (18)..(18): Xaa can be any one of F, I, L, M, T, V, W, and Y
  misc_feature (19)..(19): Xaa can be any amino acid
  misc_feature (20)..(20): Xaa can be any one of F, I, L, M, T, V, W, and Y
  misc_feature (21)..(21): Xaa can be any amino acid, or is not present if X3 is not present
  misc_feature (22)..(22): Xaa can be any one of F, I, L, M, T, V, W, and Y, or is not present if X3 is not present
  misc_feature (23)..(23): Xaa can be any amino acid, or is not present if X1 is not present
  misc_feature (24)..(24): Xaa can be any one of F, I, L, M, T, V, W, and Y, or is not present if X1 is not present
XXXXXXXXXXXNGXXXXXXXXXXX

SEQ ID NO: 2 - protein, 20 aa, Artificial Sequence
  Synthetic peptide
VLTKVKTKVNGTKVEVKVLV